European Patent Application EP 4 538 375 A1, published April 16, 2025. Title: EP6 PROMOTER, RELATED BIOMATERIAL, AND USE THEREOF. Applicant: NINGXIA EPPEN BIOTECH CO., LTD. Application CN. The sequence listing filed with the application follows.

SEQUENCE LISTING (83 sequences)

SEQ ID NO: 1 - DNA, 122 bp, Escherichia coli
  source 1..122: mol_type = genomic DNA
gaatttctccgcgtttttttcgcattcatctcgctaacttcgcttattatggggatcagtttcagggtttcaagggaagcactcacattgtcatcaatcttcgcaacaaggacctcggaaaa

SEQ ID NO: 2 - DNA, 7894 bp, Artificial sequence
  source 1..7894: mol_type = other DNA
tctagagtcgacctgcaggcatgcaagcttggctgttttggcggatgagagaagattttcagcctgatacagattaaatcagaacgcagaagcggtctgataaaacagaatttgcctggcggcagtagcgcggtggtcccacctgaccccatgccgaactcagaagtgaaacgccgtagcgccgatggtagtgtggggtctccccatgcgagagtagggaactgccaggcatcaaataaaacgaaaggctcagtcgaaagactgggcctttcgttttatctgttgtttgtcggtgaacgctctcctgagtaggacaaatccgccgggagcggatttgaacgttgcgaagcaacggcccggagggtggcgggcaggacgcccgccataaactgccaggcatcaaattaagcagaaggccatcctgacggatggcctttttgcgtttctacaaactctttttgtttatttttctaaatacattcaaatatgtatccgctcatgaattaattccgctagatgacgtgcggcttcgacctcctgggcgtggcgcttgttggcgcgctcgcggctggctgcggcacgacacgcgtctgagcagtattttgcgcgccgtcctcgtgggtcaggccggggtgggatcaggccaccgcagtaggcgcagctgatgcgatcctccactactgcgcgtcctcctggcgctgccgagcacgcagctcgtcggccagctcttcaaggtcggccacaagcgtttctaggtcgctcgcggcacttgcccagtcgcgtgatgctggcgcgtctgtcgtatcgagggcgcggaaaaatccgatcaccgtttttaaatcgacggcggcatcgagtgcgtcggactccagcgcgacatcggagagatccaccgctgatgcttcaggccagttttggtacttcgtcgtgaaggtcatgacaccattataacgaacgttcgttaaaaattctagccccaattctgataatttcttccggcactcctgcgaaaacctgcgagacttcttgcccagaaaaaacgccaagcgcagcggttaccgcactttttttccaggtgatttcaccctgaccagcgaagcggcactttagtgcatgaggtgtgcccctggtttcccctctttggagggttcaacccaaaaaagcacacaagcaaaaatgaaaatcatcatgagcaagttggtgcgaagcagcaacgcgctagctccaaaaaggtctccaggatctcgaggagatttttgagggggagggagtcgaggaagagccagagcagaaggcggggaaccgttctctgccgacagcgtgagccccccttaaaaatcaggccggggaggaaccggggagggatcagagctaggagcgagacaccctaaagggggggaaccgttttctgctgacggtgtttcgtttattagttttcagcccgtggatagcggagggtgagggcaagtgagagccagagcaaggacgggacccctaaaggggggaaccgttttctgctgacggtgtttcgtttattagttttcagcccgtggacggccgcgtttagcttccattccaagtgcctttctgacttgttggatgcgcctttcactgacacctagttcgcctgcaagctcacgagtcgagggatcagcaaccgattgagaacgggcatccaggatcgcagttttgacgcgaagttcgagcaactcgcctgtcatttctcggcgtttgtttgcttccgctaatcgctgtcgcgtctcctgcgcatacttactttctgggtcagcccatctgcgtgcattcgatgtagctgcgccccgtcgccccatcgtcgctagagctttccgccctcggctgctctgcgtttccacccgacgagcagggacgactggctggcctttagccacgtagccgcgcacacgacgcgccatcgtcaggcgatcacgcatggcgggaagatccggctcccggccgtctgcaccgaccgcctgggcaacgttgtacgccacttcatacgcgtcgatgatcttggcatcttttaggcgctcaccagcagctttgagctggtatcccacggtcaacgcgtggcgaaacgcggtctcgtcgcgcgctcgctctggatttgtccagagcactcgcacgccgtcgatcaggtcgccggacgcgtccagggcgctcggcaggctcgcgtccaaaatcgctagcgccttggcttctgcggtggcgcgttgtgccgcttcaatgcgggcgcgtccgctggaaaagtcctgctcaatgtactttttcggcttctgtgatccggtcatcgttcgagcaatctccattaggtcggccagccgatccacacgatcatgctggcagtgccatttataggctgtcggatcgtctgagacgtgcagcggccaccggctcagcctatgcgaaaaagcctggtcagcgccgaaaacacgagtcatttcttccgtcgttgcagccagcaggcgcatatttgggctggttttacctgctgcggcatacaccgggtcaatgagccagatgagctggcatttcccgctcagcggattcacgccgatccaagccggcgctttttctaggcgtgcccatttctctaaaatcgcgtagacctgcgggtttacgtgctcaatcttcccgccggcctggtggctgggcacatcgatgtcaagcacgatcaccgcggcatgttgcgcgtgcgtcagcgcaacgtactggcaccgcgtcagcgcttttgagccagcccggtagagctttggttgggtttcgccggtatccgggtttttaatccaggcgctcgcgaaatctcttgtcttgctgccctggaagctttcgcgtcccaggtgagcgagcagttcgcggcgatcttctgccgtccagccgcgtgagccgcagcgcatagcttcggggtgggtgtcgaacagatcggcggacaatttccacgcgctagctgtgactgtgtcctgcggatcggctagagtcatgtcttgagtgctttctcccagctgatgactgggggttagccgacgccctgtgagttcccgctcacggggcgttcaactttttcaggtatttgtgcagcttatcgtgttttcttcgtaaatgaacgcttaactaccttgttaaacgtggcaaataggcaggattgatggggatctagcttcacgctgccgcaagcactcagggcgcaagggctgctaaaggaagcggaacacgtagaaagccagtccgcagaaacggtgctgaccccggatgaatgtcagctactgggctatctggacaagggaaaacgcaagcgcaaagagaaagcaggtagcttgcagtgggcttacatggcgatagctagactgggcggttttatggacagcaagcgaaccggaattgccagctggggcgccctctggtaaggttgggaagccctgcaaagtaaactggatggctttcttgccgccaaggatctgatggcgcaggggatcaagatctgatcaagagacaggatgaggatcgtttcgcatgattgaacaagatggattgcacgcaggttctccggccgcttgggtggagaggctattcggctatgactgggcacaacagacaatcggctgctctgatgccgccgtgttccggctgtcagcgcaggggcgcccggttctttttgtcaagaccgacctgtccggtgccctgaatgaactccaagacgaggcagcgcggctatcgtggctggccacgacgggcgttccttgcgcagctgtgctcgacgttgtcactgaagcgggaagggactggctgctattgggcgaagtgccggggcaggatctcctgtcatctcaccttgctcctgccgagaaagtatccatcatggctgatgcaatgcggcggctgcatacgcttgatccggctacctgcccattcgaccaccaagcgaaacatcgcatcgagcgagcacgtactcggatggaagccggtcttgtcgatcaggatgatctggacgaagagcatcaggggctcgcgccagccgaactgttcgccaggctcaaggcgcggatgcccgacggcgaggatctcgtcgtgacccatggcgatgcctgcttgccgaatatcatggtggaaaatggccgcttttctggattcatcgactgtggccggctgggtgtggcggaccgctatcaggacatagcgttggctacccgtgatattgctgaagagcttggcggcgaatgggctgaccgcttcctcgtgctttacggtatcgccgctcccgattcgcagcgcatcgccttctatcgccttcttgacgagttcttctgagcgggactctggggttcgcggaatcatgaccaaaatcccttaacgtgagttttcgttccactgagcgtcagaccccgtagaaaagatcaaaggatcttcttgagatcctttttttctgcgcgtaatctgctgcttgcaaacaaaaaaaccaccgctaccagcggtggtttgtttgccggatcaagagctaccaactctttttccgaaggtaactggcttcagcagagcgcagataccaaatactgtccttctagtgtagccgtagttaggccaccacttcaagaactctgtagcaccgcctacatacctcgctctgctaatcctgttaccagtggctgctgccagtggcgataagtcgtgtcttaccgggttggactcaagacgatagttaccggataaggcgcagcggtcgggctgaacggggggttcgtgcacacagcccagcttggagcgaacgacctacaccgaactgagatacctacagcgtgagctatgagaaagcgccacgcttcccgaagggagaaaggcggacaggtatccggtaagcggcagggtcggaacaggagagcgcacgagggagcttccagggggaaacgcctggtatctttatagtcctgtcgggtttcgccacctctgacttgagcgtcgatttttgtgatgctcgtcaggggggcggagcctatggaaaaacgccagcaacgcggcctttttacggttcctggccttttgctggccttttgctcacatgttctttcctgcgttatcccctgattctgtggataaccgtattaccgcctttgagtgagctgataccgctcgccgcagccgaacgaccgagcgcagcgagtcagtgagcgaggaagcggaagagcgcctgatgcggtattttctccttacgcatctgtgcggtatttcacaccgcatatggtgcactctcagtacaatctgctctgatgccgcatagttaagccagtatacactccgctatcgctacgtgactgggtcatggctgcgccccgacacccgccaacacccgctgacgcgccctgacgggcttgtctgctcccggcatccgcttacagacaagctgtgaccgtctccgggagctgcatgtgtcagaggttttcaccgtcatcaccgaaacgcgcgaggcagcagatcaattcgcgcgcgaaggcgaagcggcatgcatttacgttgacaccatcgaatggtgcaaaacctttcgcggtatggcatgatagcgcccggaagagagtcaattcagggtggtgaatgtgaaaccagtaacgttatacgatgtcgcagagtatgccggtgtctcttatcagaccgtttcccgcgtggtgaaccaggccagccacgtttctgcgaaaacgcgggaaaaagtggaagcggcgatggcggagctgaattacattcccaaccgcgtggcacaacaactggcgggcaaacagtcgttgctgattggcgttgccacctccagtctggccctgcacgcgccgtcgcaaattgtcgcggcgattaaatctcgcgccgatcaactgggtgccagcgtggtggtgtcgatggtagaacgaagcggcgtcgaagcctgtaaagcggcggtgcacaatcttctcgcgcaacgcgtcagtgggctgatcattaactatccgctggatgaccaggatgccattgctgtggaagctgcctgcactaatgttccggcgttatttcttgatgtctctgaccagacacccatcaacagtattattttctcccatgaagacggtacgcgactgggcgtggagcatctggtcgcattgggtcaccagcaaatcgcgctgttagcgggcccattaagttctgtctcggcgcgtctgcgtctggctggctggcataaatatctcactcgcaatcaaattcagccgatagcggaacgggaaggcgactggagtgccatgtccggttttcaacaaaccatgcaaatgctgaatgagggcatcgttcccactgcgatgctggttgccaacgatcagatggcgctgggcgcaatgcgcgccattaccgagtccgggctgcgcgttggtgcggatatctcggtagtgggatacgacgataccgaagacagctcatgttatatcccgccgtcaaccaccatcaaacaggattttcgcctgctggggcaaaccagcgtggaccgcttgctgcaactctctcagggccaggcggtgaagggcaatcagctgttgcccgtctcactggtgaaaagaaaaaccaccctggcgcccaatacgcaaaccgcctctccccgcgcgttggccgattcattaatgcagctggcacgacaggtttcccgactggaaagcgggcagtgagcgcaacgcaattaatgtgagttagcgcgaattgatctggtttgacagcttatcatcgactgcacggtgcaccaatgcttctggcgtcaggcagccatcggaagctgtggtatggctgtgcaggtcgtaaatcactgcataattcgtgtcgctcaaggcgcactcccgttctggataatgttttttgcgccgacatcataacggttctggcaaatattctgaaatgagctgttgacaattaatcatccggctcgtataatgtgtggaattgtgagcggataacaatttcacacaggaaacagaccatggaattcgagctcggtacccggggatcctctaggaatttctccgcgtttttttcgcattcatctcgctaacttcgcttattatggggatcagtttcagggtttcaagggaagcactcacattgtcatcaatcttcgcaacaaggacctcggaaaaatgcgtaaaggagaagaagataacatggctatcattaaagagttcatgcgcttcaaagttcacatggagggttctgttaacggtcacgagttcgagatcgaaggcgaaggcgagggccgtccgtatgaaggcacccagaccgccaaactgaaagtgactaaaggcggcccgctgccttttgcgtgggacatcctgagcccgcaatttatgtacggttctaaagcgtatgttaaacacccagcggatatcccggactatctgaagctgtcttttccggaaggtttcaagtgggaacgcgtaatgaattttgaagatggtggtgtcgtgaccgtcactcaggactcctccctgcaggatggcgagttcatctataaagttaaactgcgtggtactaattttccatctgatggcccggtgatgcagaaaaagacgatgggttgggaggcgtctagcgaacgcatgtatccggaagatggtgcgctgaaaggcgaaattaaacagcgcctgaaactgaaagatggcggccattatgacgctgaagtgaaaaccacgtacaaagccaagaaacctgtgcagctgcctggcgcgtacaatgtgaatattaaactggacatcacctctcataatgaagattatacgatcgtagagcaatatgagcgcgcggagggtcgtcattctaccggtggcatggatgaactatacaaactagagtcgacctgcaggcatgcaagcttggctgttttggcgga

SEQ ID NO: 3 - DNA, 124 bp, Artificial sequence
  source 1..124: mol_type = other DNA
gaatttcttcgcgttttttttgcatccatcttgttaacttcgcttattatggggatcagtttccgggtttcaagggaagcggacacattgtcactatttcatttaacgcagggacctccaaatc

SEQ ID NO: 4 - DNA, 1486 bp, Corynebacterium glutamicum
  source 1..1486: mol_type = genomic DNA
tacggctccaaggacgtttgttttctgggtcagttaccccaaaaagcatatacagagaccaatgatttttcattaaaaaggcagggatttgttataagtatgggtcgtattctgtgcgacgggtgtacctcggctagaatttctccccatggctacagttgaaaatttcaatgaacttcccgcacacgtatggccacgcaatgccgtgcgccaagaagacggcgttgtcaccgtcgctggtgtgcctctgcctgacctcgctgaagaatacggaaccccactgttcgtagtcgacgaggacgatttccgttcccgctgtcgcgacatggctaccgcattcggtggaccaggcaatgtgcactacgcatctaaagcgttcctgaccaagaccattgcacgttgggttgatgaagaggggctggcactggacattgcatccatcaacgaactgggcattgccctggccgctggtttccccgccagccgtatcaccgcgcacggcaacaacaaaggcgtagagttcctgcgcgcgttggttcaaaacggtgtgggacacgtggtgctggactccgcacaggaactagaactgttggattacgttgccgctggtgaaggcaagattcaggacgtgttgatccgcgtaaagccaggcatcgaagcacacacccacgagttcatcgccactagccacgaagaccagaagttcggattctccctggcatccggttccgcattcgaagcagcaaaagccgccaacaacgcagaaaacctgaacctggttggcctgcactgccacgttggttcccaggtgttcgacgccgaaggcttcaagctggcagcagaacgcgtgttgggcctgtactcacagatccacagcgaactgggcgttgcccttcctgaactggatctcggtggcggatacggcattgcctataccgcagctgaagaaccactcaacgtcgcagaagttgcctccgacctgctcaccgcagtcggaaaaatggcagcggaactaggcatcgacgcaccaaccgtgcttgttgagcccggccgcgctatcgcaggcccctccaccgtgaccatctacgaagtcggcaccaccaaagacgtccacgtagacgacgacaaaacccgccgttacatcgccgtggacggaggcatgtccgacaacatccgcccagcactctacggctccgaatacgacgcccgcgtagtatcccgcttcgccgaaggagacccagtaagcacccgcatcgtgggctcccactgcgaatccggcgatatcctgatcaacgatgaaatctacccatctgacatcaccagcggcgacttccttgcactcgcagccaccggcgcatactgctacgccatgagctcccgctacaacgccttcacacggcccgccgtcgtgtccgtccgcgctggcagctcccgcctcatgctgcgccgcgaaacgctcgacgacatcctctcactagaggcataa

SEQ ID NO: 5 - DNA, 1648 bp, Artificial sequence
  source 1..1648: mol_type = other DNA
cagtgccaagcttgcatgcctgcaggtcgactctagcccaggtgaagaagtcgttgagggagtttttgtagccctgttcttgggaggccatgatgccgttccatgccaggctgggcgccattgcggaatcgaggacaaccttgtcggtgtgctgtgggtagcgggtggcgtagaccgatccgaggtaggttccgtaggacagtccgaagatggagatcttgtcatcgccaagtgcttggcggacgcgctcccagtcgttggcggtgttgtcggtggtcaggctggaggtgtagccgggggtgccgatctcgcaggattctttaacgaaagcgccttcgcgggtgagcagcgagaggaaatcgtatcctggtgcgatgttgtcgcagttaaccggtgtggagccgaccattccgcgaggctgcactgcaacgaggtcgtagttttggtacatggcttctggccagttcatggattggctgccgaagaagctataggcatcgccaccagggccaccggagttaccgaagatggtgccgtgcttttcgccttgggcagggaccttgacaaagcccacgctgatatcgccaagtgagggatcagaatagtgcatgggcacgtcgatgctgccacattgagcggaggcaatatctacctgaggtgggcattcttcccagcggatgttttcttgcgctgctgcagtgggcattgataccaaaaaggggctaagcgcagtcgaggcggcaagaactgctactaccctttttattgtcgaacggggcatgaatttctccgcgtttttttcgcattcatctcgctaacttcgcttattatggggatcagtttcagggtttcaagggaagcactcacattgtcatcaatcttcgcaacaaggacctcggaaaaatgacaccagctgatctcgcaacattgattaaagagaccgcggtagaggttttgacctcccgcgagctcgatacttctgttcttccggagcaggtagttgtggagcgtccgcgtaacccagagcacggcgattacgccaccaacattgcattgcaggtggctaaaaaggtcggtcagaaccctcgggatttggctacctggctggcagaggcattggctgcagatgacgccattgattctgctgaaattgctggcccaggctttttgaacattcgccttgctgcagcagcacagggtgaaattgtggccaagattctggcacagggcgagactttcggaaactccgatcacctttcccacttggacgtgaacctcgagttcgtttctgcaaacccaaccggacctattcaccttggcggaacccgctgggctgccgtgggtgactctttgggtcgtgtgctggaggcttccggcgcgaaagtgacccgcgaatactacttcaacgatcacggtcgccagatcgatcgtttcgctttgtcccttcttgcagcggcgaagggcgagccaacgccagaagacggttatggcggcgaatacattaaggaaattgcggaggcaatcgtcgaaaagcatcctgaagcgttggctttggagcctgccgcaacccaggagcttttccgcgctgaaggcgtggagatgatgttcgagggtaccgagctcgaattcgtaatcatggtcatagctg

SEQ ID NO: 6 - DNA, 1650 bp, Artificial sequence
  source 1..1650: mol_type = other DNA
cagtgccaagcttgcatgcctgcaggtcgactctagcccaggtgaagaagtcgttgagggagtttttgtagccctgttcttgggaggccatgatgccgttccatgccaggctgggcgccattgcggaatcgaggacaaccttgtcggtgtgctgtgggtagcgggtggcgtagaccgatccgaggtaggttccgtaggacagtccgaagatggagatcttgtcatcgccaagtgcttggcggacgcgctcccagtcgttggcggtgttgtcggtggtcaggctggaggtgtagccgggggtgccgatctcgcaggattctttaacgaaagcgccttcgcgggtgagcagcgagaggaaatcgtatcctggtgcgatgttgtcgcagttaaccggtgtggagccgaccattccgcgaggctgcactgcaacgaggtcgtagttttggtacatggcttctggccagttcatggattggctgccgaagaagctataggcatcgccaccagggccaccggagttaccgaagatggtgccgtgcttttcgccttgggcagggaccttgacaaagcccacgctgatatcgccaagtgagggatcagaatagtgcatgggcacgtcgatgctgccacattgagcggaggcaatatctacctgaggtgggcattcttcccagcggatgttttcttgcgctgctgcagtgggcattgataccaaaaaggggctaagcgcagtcgaggcggcaagaactgctactaccctttttattgtcgaacggggcatgaatttcttcgcgttttttttgcatccatcttgttaacttcgcttattatggggatcagtttccgggtttcaagggaagcggacacattgtcactatttcatttaacgcagggacctccaaatcatgacaccagctgatctcgcaacattgattaaagagaccgcggtagaggttttgacctcccgcgagctcgatacttctgttcttccggagcaggtagttgtggagcgtccgcgtaacccagagcacggcgattacgccaccaacattgcattgcaggtggctaaaaaggtcggtcagaaccctcgggatttggctacctggctggcagaggcattggctgcagatgacgccattgattctgctgaaattgctggcccaggctttttgaacattcgccttgctgcagcagcacagggtgaaattgtggccaagattctggcacagggcgagactttcggaaactccgatcacctttcccacttggacgtgaacctcgagttcgtttctgcaaacccaaccggacctattcaccttggcggaacccgctgggctgccgtgggtgactctttgggtcgtgtgctggaggcttccggcgcgaaagtgacccgcgaatactacttcaacgatcacggtcgccagatcgatcgtttcgctttgtcccttcttgcagcggcgaagggcgagccaacgccagaagacggttatggcggcgaatacattaaggaaattgcggaggcaatcgtcgaaaagcatcctgaagcgttggctttggagcctgccgcaacccaggagcttttccgcgctgaaggcgtggagatgatgttcgagggtaccgagctcgaattcgtaatcatggtcatagctg

SEQ ID NO: 7 - DNA, 885 bp, Artificial sequence
  source 1..885: mol_type = other DNA
ggcgacgatcttgtttgaccagttttggtacacggctagtggggtagtgccgaggccatacgtgtcgttgttttctgcaacccaggtgaagaagtcgttgagggagtttttgtagccctgttcttgggaggccatgatgccgttccatgccaggctgggcgccattgcggaatcgaggacaaccttgtcggtgtgctgtgggtagcgggtggcgtagaccgatccgaggtaggttccgtaggacagtccgaagatggagatcttgtcatcgccaagtgcttggcggacgcgctcccagtcgttggcggtgttgtcggtggtcaggctggaggtgtagccgggggtgccgatctcgcaggattctttaacgaaagcgccttcgcgggtgagcagcgagaggaaatcgtatcctggtgcgatgttgtcgcagttaaccggtgtggagccgaccattccgcgaggctgcactgcaacgaggtcgtagttttggtacatggcttctggccagttcatggattggctgccgaagaagctataggcatcgccaccagggccaccggagttaccgaagatggtgccgtgcttttcgccttgggcagggaccttgacaaagcccacgctgatatcgccaagtgagggatcagaatagtgcatgggcacgtcgatgctgccacattgagcggaggcaatatctacctgaggtgggcattcttcccagcggatgttttcttgcgctgctgcagtgggcattgataccaaaaaggggctaagcgcagtcgaggcggcaagaactgctactaccctttttattgtcgaacggggcatgaatttctccgcgtttttttcgcattcatctcgctaacttcgcttattatggggatcagt

SEQ ID NO: 8 - DNA, 885 bp, Artificial sequence
  source 1..885: mol_type = other DNA
ggcgacgatcttgtttgaccagttttggtacacggctagtggggtagtgccgaggccatacgtgtcgttgttttctgcaacccaggtgaagaagtcgttgagggagtttttgtagccctgttcttgggaggccatgatgccgttccatgccaggctgggcgccattgcggaatcgaggacaaccttgtcggtgtgctgtgggtagcgggtggcgtagaccgatccgaggtaggttccgtaggacagtccgaagatggagatcttgtcatcgccaagtgcttggcggacgcgctcccagtcgttggcggtgttgtcggtggtcaggctggaggtgtagccgggggtgccgatctcgcaggattctttaacgaaagcgccttcgcgggtgagcagcgagaggaaatcgtatcctggtgcgatgttgtcgcagttaaccggtgtggagccgaccattccgcgaggctgcactgcaacgaggtcgtagttttggtacatggcttctggccagttcatggattggctgccgaagaagctataggcatcgccaccagggccaccggagttaccgaagatggtgccgtgcttttcgccttgggcagggaccttgacaaagcccacgctgatatcgccaagtgagggatcagaatagtgcatgggcacgtcgatgctgccacattgagcggaggcaatatctacctgaggtgggcattcttcccagcggatgttttcttgcgctgctgcagtgggcattgataccaaaaaggggctaagcgcagtcgaggcggcaagaactgctactaccctttttattgtcgaacggggcatgaatttcttcgcgttttttttgcatccatcttgttaacttcgcttattatggggatcagt

SEQ ID NO: 9 - DNA, 841 bp, Artificial sequence
  source 1..841: mol_type = other DNA
cgcttattatggggatcagtttcagggtttcaagggaagcactcacattgtcatcaatcttcgcaacaaggacctcggaaaaatgacaccagctgatctcgcaacattgattaaagagaccgcggtagaggttttgacctcccgcgagctcgatacttctgttcttccggagcaggtagttgtggagcgtccgcgtaacccagagcacggcgattacgccaccaacattgcattgcaggtggctaaaaaggtcggtcagaaccctcgggatttggctacctggctggcagaggcattggctgcagatgacgccattgattctgctgaaattgctggcccaggctttttgaacattcgccttgctgcagcagcacagggtgaaattgtggccaagattctggcacagggcgagactttcggaaactccgatcacctttcccacttggacgtgaacctcgagttcgtttctgcaaacccaaccggacctattcaccttggcggaacccgctgggctgccgtgggtgactctttgggtcgtgtgctggaggcttccggcgcgaaagtgacccgcgaatactacttcaacgatcacggtcgccagatcgatcgtttcgctttgtcccttcttgcagcggcgaagggcgagccaacgccagaagacggttatggcggcgaatacattaaggaaattgcggaggcaatcgtcgaaaagcatcctgaagcgttggctttggagcctgccgcaacccaggagcttttccgcgctgaaggcgtggagatgatgttcgagcacatcaaatcttccctgcatgagttcggcaccgatttcgatgtctactac

SEQ ID NO: 10 - DNA, 843 bp, Artificial sequence
  source 1..843: mol_type = other DNA
cgcttattatggggatcagtttccgggtttcaagggaagcggacacattgtcactatttcatttaacgcagggacctccaaatcatgacaccagctgatctcgcaacattgattaaagagaccgcggtagaggttttgacctcccgcgagctcgatacttctgttcttccggagcaggtagttgtggagcgtccgcgtaacccagagcacggcgattacgccaccaacattgcattgcaggtggctaaaaaggtcggtcagaaccctcgggatttggctacctggctggcagaggcattggctgcagatgacgccattgattctgctgaaattgctggcccaggctttttgaacattcgccttgctgcagcagcacagggtgaaattgtggccaagattctggcacagggcgagactttcggaaactccgatcacctttcccacttggacgtgaacctcgagttcgtttctgcaaacccaaccggacctattcaccttggcggaacccgctgggctgccgtgggtgactctttgggtcgtgtgctggaggcttccggcgcgaaagtgacccgcgaatactacttcaacgatcacggtcgccagatcgatcgtttcgctttgtcccttcttgcagcggcgaagggcgagccaacgccagaagacggttatggcggcgaatacattaaggaaattgcggaggcaatcgtcgaaaagcatcctgaagcgttggctttggagcctgccgcaacccaggagcttttccgcgctgaaggcgtggagatgatgttcgagcacatcaaatcttccctgcatgagttcggcaccgatttcgatgtctactac

SEQ ID NO: 11 - DNA, 1161 bp, Corynebacterium glutamicum
  source 1..1161: mol_type = genomic DNA
ccccctctttaaggacagaaaggtttcaaccaagacatgttcgagctaatcgacgactggggtcccgaaaagatcgtcatcgtcagcgatcaaaaaaccgggatgcgtggcgtacttgtcatcgacaacaccgcccgcggcatgggcaagggcggcacgcgcatgcagcccaccgtttcagtcgcagaaatagccaggttggctcgcgtcatgacctggaaatgggctggtgtagacctcttttatggtggtgcaaaagccggaatccaagcagaccccacctccccagataaagaagcaatccttcggtcattcgtcagaaaactctccaacgaagtacctaaagaatatgtcttcggcctggacatggggctgactgaaaatgacgccgccatcatcgtcgacgagctcggctggggcaccagtatgggaacaccctacgagctcggtggagtgccctacgacaagcttggtatcaccggctttggtgttgcagaagtggtggatcaagtagcacaaatgcaaaaactcaaaggtgcatcggtagcagtccaaggcttcggtgccgttggacatgccacagcttcccgcctggcagaacttggctatcctgttgtggctatctccacagcaaagggagcaatcgcagaccccaacgggctcaacatccccgagctcatggaactacgcgatcaggtgggtgactcacttgtggaccactacccagcacttcgcatcaacccaggtgacgaacttttcaccgaagccgaaatcctcgtaccggcagcgctccaggacgtcatcgatgaagacgcagccaatcgactacaagcacaactcgtcgtcgaaggagcaaaccttcccactaatgaagccgcacaaaaagtcctaagtaaccgtggcatcactgtggttccagactttgtcgccaacgccggaggagtagtcgccgcagcattcgccatggataaccgcatgtctgcattccgtgcagagactgccaacatcttcacgagcgtttccgacaaactccgatccaatgccgaaactgtcctgaatttcacctctgaatctgacctgaccagccacgaagcggcaaggcaactttcacaggaacgagttcttgcagctatgcgcgccagaggtatggttcgccgataa

SEQ ID NO: 12 - DNA, 1699 bp, Artificial sequence
  source 1..1699: mol_type = other DNA
cagtgccaagcttgcatgcctgcaggtcgactctagcggaaacaacgcagccatagtcaccccagatgcagatcttgacctggcacttcgcggaattgtcttcgcggctgccggaaccgctggtcagcgctgcaccaccatgcgccgcgttatcgtccacgagtccattgcagaagagctcaccgaaaaactcgtttccgcataccaaaccctgaccatcggcgatcctcgcgacgagcagatcctcgttggaccactgatcaatgaatccggattccagggtatgcaggatgcactcaaggctgcaaccgaacagggcggaacggttatcaccggtggcaaccgagtcctcgaagatgaattcccagaggcctactacgttgagcctgcaatcgtaaccatgccagcacaaacagacattgtgcgcgatgaaaccttcgcaccaattctctacgtgctgacctactccactttggaagaagcaatcgcactccaaaacgatgttccacagggcctttcttctgcaatcttcaccgaaaaccagcgcgaagcagagctcttcgtctccgcttccggctccgactgtggcattgccaacgtcaacatcggtacctccggcgcagaaatcggcggcgcattcggtggcgaaaaggaaaccggtggcggacgcgaatccggctccgactcctggaagtcctacatgcgacgcgccaccaacaccgtcaactactccggcgaactgccactcgcccaaggcgttaaattcctctaagaatttctccgcgtttttttcgcattcatctcgctaacttcgcttattatggggatcagtttcagggtttcaagggaagcactcacattgtcatcaatcttcgcaacaaggacctcggaaaaatgttcgagctaatcgacgactggggtcccgaaaagatcgtcatcgtcagcgatcaaaaaaccgggatgcgtggcgtacttgtcatcgacaacaccgcccgcggcatgggcaagggcggcacgcgcatgcagcccaccgtttcagtcgcagaaatagccaggttggctcgcgtcatgacctggaaatgggctggtgtagacctcttttatggtggtgcaaaagccggaatccaagcagaccccacctccccagataaagaagcaatccttcggtcattcgtcagaaaactctccaacgaagtacctaaagaatatgtcttcggcctggacatggggctgactgaaaatgacgccgccatcatcgtcgacgagctcggctggggcaccagtatgggaacaccctacgagctcggtggagtgccctacgacaagcttggtatcaccggctttggtgttgcagaagtggtggatcaagtagcacaaatgcaaaaactcaaaggtgcatcggtagcagtccaaggcttcggtgccgttggacatgccacagcttcccgcctggcagaacttggctatcctgttgtggctatctccacagcaaagggagcaatcgcagaccccaacgggctcaacatccccgagctcatggaactacgcgatcaggtgggtgactcacttgtggaccactacccagcacttcgcatcaacccaggtgacgaacttttcaccgaagccgaaatcctcgtaccggcagcgctccaggacgtcatgggtaccgagctcgaattcgtaatcatggtcatagctg

SEQ ID NO: 13 - DNA, 1701 bp, Artificial sequence
  source 1..1701: mol_type = other DNA
cagtgccaagcttgcatgcctgcaggtcgactctagcggaaacaacgcagccatagtcaccccagatgcagatcttgacctggcacttcgcggaattgtcttcgcggctgccggaaccgctggtcagcgctgcaccaccatgcgccgcgttatcgtccacgagtccattgcagaagagctcaccgaaaaactcgtttccgcataccaaaccctgaccatcggcgatcctcgcgacgagcagatcctcgttggaccactgatcaatgaatccggattccagggtatgcaggatgcactcaaggctgcaaccgaacagggcggaacggttatcaccggtggcaaccgagtcctcgaagatgaattcccagaggcctactacgttgagcctgcaatcgtaaccatgccagcacaaacagacattgtgcgcgatgaaaccttcgcaccaattctctacgtgctgacctactccactttggaagaagcaatcgcactccaaaacgatgttccacagggcctttcttctgcaatcttcaccgaaaaccagcgcgaagcagagctcttcgtctccgcttccggctccgactgtggcattgccaacgtcaacatcggtacctccggcgcagaaatcggcggcgcattcggtggcgaaaaggaaaccggtggcggacgcgaatccggctccgactcctggaagtcctacatgcgacgcgccaccaacaccgtcaactactccggcgaactgccactcgcccaaggcgttaaattcctctaagaatttcttcgcgttttttttgcatccatcttgttaacttcgcttattatggggatcagtttccgggtttcaagggaagcggacacattgtcactatttcatttaacgcagggacctccaaatcatgttcgagctaatcgacgactggggtcccgaaaagatcgtcatcgtcagcgatcaaaaaaccgggatgcgtggcgtacttgtcatcgacaacaccgcccgcggcatgggcaagggcggcacgcgcatgcagcccaccgtttcagtcgcagaaatagccaggttggctcgcgtcatgacctggaaatgggctggtgtagacctcttttatggtggtgcaaaagccggaatccaagcagaccccacctccccagataaagaagcaatccttcggtcattcgtcagaaaactctccaacgaagtacctaaagaatatgtcttcggcctggacatggggctgactgaaaatgacgccgccatcatcgtcgacgagctcggctggggcaccagtatgggaacaccctacgagctcggtggagtgccctacgacaagcttggtatcaccggctttggtgttgcagaagtggtggatcaagtagcacaaatgcaaaaactcaaaggtgcatcggtagcagtccaaggcttcggtgccgttggacatgccacagcttcccgcctggcagaacttggctatcctgttgtggctatctccacagcaaagggagcaatcgcagaccccaacgggctcaacatccccgagctcatggaactacgcgatcaggtgggtgactcacttgtggaccactacccagcacttcgcatcaacccaggtgacgaacttttcaccgaagccgaaatcctcgtaccggcagcgctccaggacgtcatgggtaccgagctcgaattcgtaatcatggtcatagctg

SEQ ID NO: 14 - DNA, 849 bp, Artificial sequence
  source 1..849: mol_type = other DNA
gaagtaggtcctcgtgttgctgcccgattcggcaaaaccatcctggagctgggcggaaacaacgcagccatagtcaccccagatgcagatcttgacctggcacttcgcggaattgtcttcgcggctgccggaaccgctggtcagcgctgcaccaccatgcgccgcgttatcgtccacgagtccattgcagaagagctcaccgaaaaactcgtttccgcataccaaaccctgaccatcggcgatcctcgcgacgagcagatcctcgttggaccactgatcaatgaatccggattccagggtatgcaggatgcactcaaggctgcaaccgaacagggcggaacggttatcaccggtggcaaccgagtcctcgaagatgaattcccagaggcctactacgttgagcctgcaatcgtaaccatgccagcacaaacagacattgtgcgcgatgaaaccttcgcaccaattctctacgtgctgacctactccactttggaagaagcaatcgcactccaaaacgatgttccacagggcctttcttctgcaatcttcaccgaaaaccagcgcgaagcagagctcttcgtctccgcttccggctccgactgtggcattgccaacgtcaacatcggtacctccggcgcagaaatcggcggcgcattcggtggcgaaaaggaaaccggtggcggacgcgaatccggctccgactcctggaagtcctacatgcgacgcgccaccaacaccgtcaactactccggcgaactgccactcgcccaaggcgttaaattcctctaagaatttctccgcgtttttttcgcattcatctcgctaacttcgcttattatggggatcagt

SEQ ID NO: 15 - DNA, 849 bp, Artificial sequence
  source 1..849: mol_type = other DNA
gaagtaggtcctcgtgttgctgcccgattcggcaaaaccatcctggagctgggcggaaacaacgcagccatagtcaccccagatgcagatcttgacctggcacttcgcggaattgtcttcgcggctgccggaaccgctggtcagcgctgcaccaccatgcgccgcgttatcgtccacgagtccattgcagaagagctcaccgaaaaactcgtttccgcataccaaaccctgaccatcggcgatcctcgcgacgagcagatcctcgttggaccactgatcaatgaatccggattccagggtatgcaggatgcactcaaggctgcaaccgaacagggcggaacggttatcaccggtggcaaccgagtcctcgaagatgaattcccagaggcctactacgttgagcctgcaatcgtaaccatgccagcacaaacagacattgtgcgcgatgaaaccttcgcaccaattctctacgtgctgacctactccactttggaagaagcaatcgcactccaaaacgatgttccacagggcctttcttctgcaatcttcaccgaaaaccagcgcgaagcagagctcttcgtctccgcttccggctccgactgtggcattgccaacgtcaacatcggtacctccggcgcagaaatcggcggcgcattcggtggcgaaaaggaaaccggtggcggacgcgaatccggctccgactcctggaagtcctacatgcgacgcgccaccaacaccgtcaactactccggcgaactgccactcgcccaaggcgttaaattcctctaagaatttcttcgcgttttttttgcatccatcttgttaacttcgcttattatggggatcagt

SEQ ID NO: 16 - DNA, 889 bp, Artificial sequence
  source 1..889: mol_type = other DNA
cgcttattatggggatcagtttcagggtttcaagggaagcactcacattgtcatcaatcttcgcaacaaggacctcggaaaaatgttcgagctaatcgacgactggggtcccgaaaagatcgtcatcgtcagcgatcaaaaaaccgggatgcgtggcgtacttgtcatcgacaacaccgcccgcggcatgggcaagggcggcacgcgcatgcagcccaccgtttcagtcgcagaaatagccaggttggctcgcgtcatgacctggaaatgggctggtgtagacctcttttatggtggtgcaaaagccggaatccaagcagaccccacctccccagataaagaagcaatccttcggtcattcgtcagaaaactctccaacgaagtacctaaagaatatgtcttcggcctggacatggggctgactgaaaatgacgccgccatcatcgtcgacgagctcggctggggcaccagtatgggaacaccctacgagctcggtggagtgccctacgacaagcttggtatcaccggctttggtgttgcagaagtggtggatcaagtagcacaaatgcaaaaactcaaaggtgcatcggtagcagtccaaggcttcggtgccgttggacatgccacagcttcccgcctggcagaacttggctatcctgttgtggctatctccacagcaaagggagcaatcgcagaccccaacgggctcaacatccccgagctcatggaactacgcgatcaggtgggtgactcacttgtggaccactacccagcacttcgcatcaacccaggtgacgaacttttcaccgaagccgaaatcctcgtaccggcagcgctccaggacgtcatcgatgaagacgcagccaatcgactacaagcacaactcgtc

SEQ ID NO: 17 - DNA, 891 bp, Artificial sequence
  source 1..891: mol_type = other DNA
cgcttattatggggatcagtttccgggtttcaagggaagcggacacattgtcactatttcatttaacgcagggacctccaaatcatgttcgagctaatcgacgactggggtcccgaaaagatcgtcatcgtcagcgatcaaaaaaccgggatgcgtggcgtacttgtcatcgacaacaccgcccgcggcatgggcaagggcggcacgcgcatgcagcccaccgtttcagtcgcagaaatagccaggttggctcgcgtcatgacctggaaatgggctggtgtagacctcttttatggtggtgcaaaagccggaatccaagcagaccccacctccccagataaagaagcaatccttcggtcattcgtcagaaaactctccaacgaagtacctaaagaatatgtcttcggcctggacatggggctgactgaaaatgacgccgccatcatcgtcgacgagctcggctggggcaccagtatgggaacaccctacgagctcggtggagtgccctacgacaagcttggtatcaccggctttggtgttgcagaagtggtggatcaagtagcacaaatgcaaaaactcaaaggtgcatcggtagcagtccaaggcttcggtgccgttggacatgccacagcttcccgcctggcagaacttggctatcctgttgtggctatctccacagcaaagggagcaatcgcagaccccaacgggctcaacatccccgagctcatggaactacgcgatcaggtgggtgactcacttgtggaccactacccagcacttcgcatcaacccaggtgacgaacttttcaccgaagccgaaatcctcgtaccggcagcgctccaggacgtcatcgatgaagacgcagccaatcgactacaagcacaactcgtc

SEQ ID NO: 18 - DNA, 1196 bp, Corynebacterium glutamicum
  source 1..1196: mol_type = genomic DNA
acagcaattaatctgattgcacctgctgcataaatgtgactagtcaaacaccgtctaattgcatgtgtgtggtagaacaataatgtagttgtctgcccaagcgagtttaactcccacgatttacagtgggggcagacatcttttcaccaaaatttttacgaaaggcgagattttctcccatggctattgaactgctttatgatgctgacgctgacctctccttgatccagggccgcaaggttgccatcgttggctacggctcccagggccacgcacactcccagaacctccgcgattctggcgttgaggttgtcattggtctgcgcgagggctccaagtccgcagagaaggcaaaggaagcaggcttcgaggtcaagaccaccgctgaggctgcagcttgggctgacgtcatcatgctcctggctccagacacctcccaggcagaaatcttcaccaacgacatcgagccaaacctgaacgcaggcgacgcactgctgttcggccacggcctgaacattcacttcgacctgatcaagccagctgacgacatcatcgttggcatggttgcgccaaagggcccaggccacttggttcgccgtcagttcgttgatggcaagggtgttccttgcctcatcgcagtcgaccaggacccaaccggaaccgcacaggctctgaccctgtcctacgcagcagcaatcggtggcgcacgcgcaggcgttatcccaaccaccttcgaagctgagaccgtcaccgacctcttcggcgagcaggctgttctctgcggtggcaccgaggaactggtcaaggttggcttcgaggttctcaccgaagctggctacgagccagagatggcatacttcgaggttcttcacgagctcaagctcatcgttgacctcatgttcgaaggtggcatcagcaacatgaactactctgtttctgacaccgctgagttcggtggctacctctccggcccacgcgtcatcgatgcagacaccaagtcccgcatgaaggacatcctgaccgatatccaggacggcaccttcaccaagcgcctcatcgcaaacgttgagaacggcaacaccgaacttgagggccttcgtgcttcctacaacaaccacccaatcgaggagaccggcgctaagctccgcgacctcatgagctgggtcaaggttgacgctcgcgcagaaaccgcttaa

SEQ ID NO: 19 - DNA, 1822 bp, Artificial sequence
  source 1..1822: mol_type = other DNA
cagtgccaagcttgcatgcctgcaggtcgactctagagagatcaacgaccgcccagtagtcatcgacttcatcgtcggtgaagacgcacaggtatggccaatggtgtctgctggatcatccaactccgatatccagtacgcactcggattgcgcccattctttgatggtgatgaatctgcagcagaagatcctgccgacattcacgaagccgtcagcgacattgatgccgccgttgaatcgaccgaggcataaggagagacccaagatggctaattctgacgtcacccgccacatcctgtccgtactcgttcaggacgtagacggaatcatttcccgcgtatcaggtatgttcacccgacgcgcattcaacctcgtgtccctcgtgtctgcaaagaccgaaacactcggcatcaaccgcatcacggttgttgtcgacgccgacgagctcaacattgagcagatcaccaagcagctcaacaagctgatccccgtgctcaaagtcgtgcgacttgatgaagagaccaccatcgcccgcgcaatcatgctggttaaggtctctgcggatagcaccaaccgtccgcagatcgtcgacgccgcgaacatcttccgcgcccgagtcgtcgacgtggctccagactctgtggttattgaatccacaggcaccccaggcaagctccgcgcactgcttgatgtgatggaaccattcggaatccgcgaactgatccaatccggacagattgcactcaaccgcggtccgaagaccatggctccggccaagatctaagaatttctccgcgtttttttcgcattcatctcgctaacttcgcttattatggggatcagtttcagggtttcaagggaagcactcacattgtcatcaatcttcgcaacaaggacctcggaaaaatggctattgaactgctttatgatgctgacgctgacctctccttgatccagggccgcaaggttgccatcgttggctacggctcccagggccacgcacactcccagaacctccgcgattctggcgttgaggttgtcattggtctgcgcgagggctccaagtccgcagagaaggcaaaggaagcaggcttcgaggtcaagaccaccgctgaggctgcagcttgggctgacgtcatcatgctcctggctccagacacctcccaggcagaaatcttcaccaacgacatcgagccaaacctgaacgcaggcgacgcactgctgttcggccacggcctgaacattcacttcgacctgatcaagccagctgacgacatcatcgttggcatggttgcgccaaagggcccaggccacttggttcgccgtcagttcgttgatggcaagggtgttccttgcctcatcgcagtcgaccaggacccaaccggaaccgcacaggctctgaccctgtcctacgcagcagcaatcggtggcgcacgcgcaggcgttatcccaaccaccttcgaagctgagaccgtcaccgacctcttcggcgagcaggctgttctctgcggtggcaccgaggaactggtcaaggttggcttcgaggttctcaccgaagctggctacgagccagagatggcatacttcgaggttcttcacgagctcaagctcatcgttgacctcatgttcgaaggtggcatcagcaacatgaactactctgtttctgacaccgctgagttcggtggctacctctccggcccacgcgtcatcgatgcagacaccaagtcccgcatgaaggacatcctgaccgatatccaggacggcaccttcaccaagcgcctcagggtaccgagctcgaattcgtaatcatggtcatagctg

SEQ ID NO: 20 - DNA, 1824 bp, Artificial sequence
  source 1..1824: mol_type = other DNA
cagtgccaagcttgcatgcctgcaggtcgactctagagagatcaacgaccgcccagtagtcatcgacttcatcgtcggtgaagacgcacaggtatggccaatggtgtctgctggatcatccaactccgatatccagtacgcactcggattgcgcccattctttgatggtgatgaatctgcagcagaagatcctgccgacattcacgaagccgtcagcgacattgatgccgccgttgaatcgaccgaggcataaggagagacccaagatggctaattctgacgtcacccgccacatcctgtccgtactcgttcaggacgtagacggaatcatttcccgcgtatcaggtatgttcacccgacgcgcattcaacctcgtgtccctcgtgtctgcaaagaccgaaacactcggcatcaaccgcatcacggttgttgtcgacgccgacgagctcaacattgagcagatcaccaagcagctcaacaagctgatccccgtgctcaaagtcgtgcgacttgatgaagagaccaccatcgcccgcgcaatcatgctggttaaggtctctgcggatagcaccaaccgtccgcagatcgtcgacgccgcgaacatcttccgcgcccgagtcgtcgacgtggctccagactctgtggttattgaatccacaggcaccccaggcaagctccgcgcactgcttgatgtgatggaaccattcggaatccgcgaactgatccaatccggacagattgcactcaaccgcggtccgaagaccatggctccggccaagatctaagaatttcttcgcgttttttttgcatccatcttgttaacttcgcttattatggggatcagtttccgggtttcaagggaagcggacacattgtcactatttcatttaacgcagggacctccaaatcatggctattgaactgctttatgatgctgacgctgacctctccttgatccagggccgcaaggttgccatcgttggctacggctcccagggccacgcacactcccagaacctccgcgattctggcgttgaggttgtcattggtctgcgcgagggctccaagtccgcagagaaggcaaaggaagcaggcttcgaggtcaagaccaccgctgaggctgcagcttgggctgacgtcatcatgctcctggctccagacacctcccaggcagaaatcttcaccaacgacatcgagccaaacctgaacgcaggcgacgcactgctgttcggccacggcctgaacattcacttcgacctgatcaagccagctgacgacatcatcgttggcatggttgcgccaaagggcccaggccacttggttcgccgtcagttcgttgatggcaagggtgttccttgcctcatcgcagtcgaccaggacccaaccggaaccgcacaggctctgaccctgtcctacgcagcagcaatcggtggcgcacgcgcaggcgttatcccaaccaccttcgaagctgagaccgtcaccgacctcttcggcgagcaggctgttctctgcggtggcaccgaggaactggtcaaggttggcttcgaggttctcaccgaagctggctacgagccagagatggcatacttcgaggttcttcacgagctcaagctcatcgttgacctcatgttcgaaggtggcatcagcaacatgaactactctgtttctgacaccgctgagttcggtggctacctctccggcccacgcgtcatcgatgcagacaccaagtcccgcatgaaggacatcctgaccgatatccaggacggcaccttcaccaagcgcctcagggtaccgagctcgaattcgtaatcatggtcatagctg

SEQ ID NO: 21 - DNA, 901 bp, Artificial sequence
  source 1..901: mol_type = other DNA
cccgactttgttaccctttctgagggacttggctgtgttgccatccgcgtcaccaaagcggaggaagtactgccagccatccaaaaggctcgagagatcaacgaccgcccagtagtcatcgacttcatcgtcggtgaagacgcacaggtatggccaatggtgtctgctggatcatccaactccgatatccagtacgcactcggattgcgcccattctttgatggtgatgaatctgcagcagaagatcctgccgacattcacgaagccgtcagcgacattgatgccgccgttgaatcgaccgaggcataaggagagacccaagatggctaattctgacgtcacccgccacatcctgtccgtactcgttcaggacgtagacggaatcatttcccgcgtatcaggtatgttcacccgacgcgcattcaacctcgtgtccctcgtgtctgcaaagaccgaaacactcggcatcaaccgcatcacggttgttgtcgacgccgacgagctcaacattgagcagatcaccaagcagctcaacaagctgatccccgtgctcaaagtcgtgcgacttgatgaagagaccaccatcgcccgcgcaatcatgctggttaaggtctctgcggatagcaccaaccgtccgcagatcgtcgacgccgcgaacatcttccgcgcccgagtcgtcgacgtggctccagactctgtggttattgaatccacaggcaccccaggcaagctccgcgcactgcttgatgtgatggaaccattcggaatccgcgaactgatccaatccggacagattgcactcaaccgcggtccgaagaccatggctccggccaagatctaagaatttctccgcgtttttttcgcattcatctcgctaacttcgcttattatggggatcagt

SEQ ID NO: 22 - DNA, 901 bp, Artificial sequence
  source 1..901: mol_type = other DNA
cccgactttgttaccctttctgagggacttggctgtgttgccatccgcgtcaccaaagcggaggaagtactgccagccatccaaaaggctcgagagatcaacgaccgcccagtagtcatcgacttcatcgtcggtgaagacgcacaggtatggccaatggtgtctgctggatcatccaactccgatatccagtacgcactcggattgcgcccattctttgatggtgatgaatctgcagcagaagatcctgccgacattcacgaagccgtcagcgacattgatgccgccgttgaatcgaccgaggcataaggagagacccaagatggctaattctgacgtcacccgccacatcctgtccgtactcgttcaggacgtagacggaatcatttcccgcgtatcaggtatgttcacccgacgcgcattcaacctcgtgtccctcgtgtctgcaaagaccgaaacactcggcatcaaccgcatcacggttgttgtcgacgccgacgagctcaacattgagcagatcaccaagcagctcaacaagctgatccccgtgctcaaagtcgtgcgacttgatgaagagaccaccatcgcccgcgcaatcatgctggttaaggtctctgcggatagcaccaaccgtccgcagatcgtcgacgccgcgaacatcttccgcgcccgagtcgtcgacgtggctccagactctgtggttattgaatccacaggcaccccaggcaagctccgcgcactgcttgatgtgatggaaccattcggaatccgcgaactgatccaatccggacagattgcactcaaccgcggtccgaagaccatggctccggccaagatctaagaatttcttcgcgttttttttgcatccatcttgttaacttcgcttattatggggatcagt

SEQ ID NO: 23 - DNA, 1023 bp, Artificial sequence
  source 1..1023: mol_type = other DNA
cgcttattatggggatcagtttcagggtttcaagggaagcactcacattgtcatcaatcttcgcaacaaggacctcggaaaaatggctattgaactgctttatgatgctgacgctgacctctccttgatccagggccgcaaggttgccatcgttggctacggctcccagggccacgcacactcccagaacctccgcgattctggcgttgaggttgtcattggtctgcgcgagggctccaagtccgcagagaaggcaaaggaagcaggcttcgaggtcaagaccaccgctgaggctgcagcttgggctgacgtcatcatgctcctggctccagacacctcccaggcagaaatcttcaccaacgacatcgagccaaacctgaacgcaggcgacgcactgctgttcggccacggcctgaacattcacttcgacctgatcaagccagctgacgacatcatcgttggcatggttgcgccaaagggcccaggccacttggttcgccgtcagttcgttgatggcaagggtgttccttgcctcatcgcagtcgaccaggacccaaccggaaccgcacaggctctgaccctgtcctacgcagcagcaatcggtggcgcacgcgcaggcgttatcccaaccaccttcgaagctgagaccgtcaccgacctcttcggcgagcaggctgttctctgcggtggcaccgaggaactggtcaaggttggcttcgaggttctcaccgaagctggctacgagccagagatggcatacttcgaggttcttcacgagctcaagctcatcgttgacctcatgttcgaaggtggcatcagcaacatgaactactctgtttctgacaccgctgagttcggtggctacctctccggcccacgcgtcatcgatgcagacaccaagtcccgcatgaaggacatcctgaccgatatccaggacggcaccttcaccaagcgcctcatcgcaaacgttgagaacggcaacaccgaacttgagggccttcgtgcttcctacaacaaccaccc

SEQ ID NO: 24 - DNA, 1025 bp, Artificial sequence
  source 1..1025: mol_type = other DNA
cgcttattatggggatcagtttccgggtttcaagggaagcggacacattgtcactatttcatttaacgcagggacctccaaatcatggctattgaactgctttatgatgctgacgctgacctctccttgatccagggccgcaaggttgccatcgttggctacggctcccagggccacgcacactcccagaacctccgcgattctggcgttgaggttgtcattggtctgcgcgagggctccaagtccgcagagaaggcaaaggaagcaggcttcgaggtcaagaccaccgctgaggctgcagcttgggctgacgtcatcatgctcctggctccagacacctcccaggcagaaatcttcaccaacgacatcgagccaaacctgaacgcaggcgacgcactgctgttcggccacggcctgaacattcacttcgacctgatcaagccagctgacgacatcatcgttggcatggttgcgccaaagggcccaggccacttggttcgccgtcagttcgttgatggcaagggtgttccttgcctcatcgcagtcgaccaggacccaaccggaaccgcacaggctctgaccctgtcctacgcagcagcaatcggtggcgcacgcgcaggcgttatcccaaccaccttcgaagctgagaccgtcaccgacctcttcggcgagcaggctgttctctgcggtggcaccgaggaactggtcaaggttggcttcgaggttctcaccgaagctggctacgagccagagatggcatacttcgaggttcttcacgagctcaagctcatcgttgacctcatgttcgaaggtggcatcagcaacatgaactactctgtttctgacaccgctgagttcggtggctacctctccggcccacgcgtcatcgatgcagacaccaagtcccgcatgaaggacatcctgaccgatatccaggacggcaccttcaccaagcgcctcatcgcaaacgttgagaacggcaacaccgaacttgagggccttcgtgcttcctacaacaaccaccc

SEQ ID NO: 25 - DNA, 84 bp, synthetic construct
  source 1..84: mol_type = other DNA
gctcaacccttaccggtcggctctaagccggcggcgtatggtaagctctgttatgtatagtccgagcacggcgaaaggatactc

SEQ ID NO: 26 - DNA, 21 bp, synthetic construct
  source 1..21: mol_type = other DNA
ggatctagagtcgacctgcag

SEQ ID NO: 27 - DNA, 25 bp, synthetic construct
  source 1..25: mol_type = other DNA
ttaactagtattgcgttgcgctcac

SEQ ID NO: 28 - DNA, 27 bp, synthetic construct
  source 1..27: mol_type = other DNA
caatactagttaatgtgagttagcgcg

SEQ ID NO: 29 - DNA, 68 bp, synthetic construct
  source 1..68: mol_type = other DNA
agagcttaccatacgccgccggcttagagccgaccggtaagggttgagcctagaggatccccgggtac

SEQ ID NO: 30 - DNA, 75 bp, synthetic construct
  source 1..75: mol_type = other DNA
gcgtatggtaagctctgttatgttatgtatagtccgagcacggcgaaaggatactcatgcgtaaaggagaagaag

SEQ ID NO: 31 - DNA, 25 bp, synthetic construct
  source 1..25: mol_type = other DNA
cgactctagatccgccaaaacagcc

SEQ ID NO: 32 - DNA, 24 bp, synthetic construct
  source 1..24: mol_type = other DNA
atgcgtaaaggagaagaagataac

SEQ ID NO: 33 - DNA, 19 bp, synthetic construct
  source 1..19: mol_type = other DNA
ctagaggatccccgggtac

SEQ ID NO: 34 - DNA, 56 bp, synthetic construct
  source 1..56: mol_type = other DNA
catggaattcgagctcggtacccggggatcctctaggaatttctccgcgttttttt

SEQ ID NO: 35 - DNA, 56 bp, synthetic construct
  source 1..56: mol_type = other DNA
aatgatagccatgttatcttcttctcctttacgcatttttccgaggtccttgttgc

SEQ ID NO: 36 - DNA, 19 bp, synthetic construct
  source 1..19: mol_type = other DNA
gtacccggggatcctctag

SEQ ID NO: 37 - DNA, 24 bp, synthetic construct
  source 1..24: mol_type = other DNA
gttatcttcttctcctttacgcat

SEQ ID NO: 38 - DNA, 56 bp, synthetic construct
  source 1..56: mol_type = other DNA
catggaattcgagctcggtacccggggatcctctaggaatttcttcgcgttttttt

SEQ ID NO: 39 - DNA, 56 bp, synthetic construct
  source 1..56: mol_type = other DNA
aatgatagccatgttatcttcttctcctttacgcatgatttggaggtccctgcgtt

SEQ ID NO: 40 - DNA, 56 bp, synthetic construct
  source 1..56: mol_type = other DNA
cagtgccaagcttgcatgcctgcaggtcgactctagcccaggtgaagaagtcgttg

SEQ ID NO: 41 - DNA, 40 bp, synthetic construct
  source 1..40: mol_type = other DNA
aaaaaaacgcggagaaattcatgccccgttcgacaataaa

SEQ ID NO: 42 - DNA, 40 bp, synthetic construct
  source 1..40: mol_type = other DNA
tttattgtcgaacggggcatgaatttctccgcgttttttt

SEQ ID NO: 43 - DNA, 40 bp, synthetic construct
  source 1..40: mol_type = other DNA
gcgagatcagctggtgtcatttttccgaggtccttgttgc

SEQ ID NO: 44 - DNA, 40 bp, synthetic construct
  source 1..40: mol_type = other DNA
gcaacaaggacctcggaaaaatgacaccagctgatctcgc

SEQ ID NO: 45 - DNA, 58 bp, synthetic construct
  source 1..58: mol_type = other DNA
cagctatgaccatgattacgaattcgagctcggtaccctcgaacatcatctccacgcc

SEQ ID NO: 46 - DNA, 40 bp, synthetic construct
  source 1..40: mol_type = other DNA
aaaaaaacgcgaagaaattcatgccccgttcgacaataaa

SEQ ID NO: 47 - DNA, 40 bp, synthetic construct
  source 1..40: mol_type = other DNA
tttattgtcgaacggggcatgaatttcttcgcgttttttt

SEQ ID NO: 48 - DNA, 40 bp, synthetic construct
  source 1..40: mol_type = other DNA
gcgagatcagctggtgtcatgatttggaggtccctgcgtt

SEQ ID NO: 49 - DNA, 40 bp, synthetic construct
  source 1..40: mol_type = other DNA
aacgcagggacctccaaatcatgacaccagctgatctcgc

SEQ ID NO: 50 - DNA, 18 bp, synthetic construct
  source 1..18: mol_type = other DNA
tgtaaaacgacggccagt

SEQ ID NO: 51 - DNA, 18 bp, synthetic construct
  source 1..18: mol_type = other DNA
caggaaacagctatgacc

SEQ ID NO: 52 - DNA, 20 bp, synthetic construct
  source 1..20: mol_type = other DNA
ggcgacgatcttgtttgacc

SEQ ID NO: 53 - DNA, 20 bp, synthetic construct
  source 1..20: mol_type = other DNA
actgatccccataataagcg

SEQ ID NO: 54 - DNA, 20 bp, synthetic construct
  source 1..20: mol_type = other DNA
cgcttattatggggatcagt

SEQ ID NO: 55 - DNA, 20 bp, synthetic construct
  source 1..20: mol_type = other DNA
gtagtagacatcgaaatcgg

SEQ ID NO: 56 - DNA, 56 bp, synthetic construct
  source 1..56: mol_type = other DNA
cagtgccaagcttgcatgcctgcaggtcgactctagcggaaacaacgcagccatag

SEQ ID NO: 57 - DNA, 40 bp, synthetic construct
  source 1..40: mol_type = other DNA
aaaaaaacgcggagaaattcttagaggaatttaacgcctt

SEQ ID NO: 58 - DNA, 40 bp, synthetic construct
  source 1..40: mol_type = other DNA
aaggcgttaaattcctctaagaatttctccgcgttttttt

SEQ ID NO: 59 - DNA, 40 bp, synthetic construct
  source 1..40: mol_type = other DNA
tcgtcgattagctcgaacatttttccgaggtccttgttgc

SEQ ID NO: 60 - DNA, 40 bp, synthetic construct
  source 1..40: mol_type = other DNA
gcaacaaggacctcggaaaaatgttcgagctaatcgacga

SEQ ID NO: 61 - DNA, 58 bp, synthetic construct
  source 1..58: mol_type = other DNA
cagctatgaccatgattacgaattcgagctcggtacccatgacgtcctggagcgctgc

SEQ ID NO: 62 - DNA, 40 bp, synthetic construct
  source 1..40: mol_type = other DNA
aaaaaaacgcgaagaaattcttagaggaatttaacgcctt

SEQ ID NO: 63 - DNA, 40 bp, synthetic construct
  source 1..40: mol_type = other DNA
aaggcgttaaattcctctaagaatttcttcgcgttttttt

SEQ ID NO: 64 - DNA, 40 bp, synthetic construct
  source 1..40: mol_type = other DNA
tcgtcgattagctcgaacatgatttggaggtccctgcgtt

SEQ ID NO: 65 - DNA, 40 bp, synthetic construct
  source 1..40: mol_type = other DNA
aacgcagggacctccaaatcatgttcgagctaatcgacga

SEQ ID NO: 66 - DNA, 20 bp, synthetic construct
  source 1..20: mol_type = other DNA
gaagtaggtcctcgtgttgc

SEQ ID NO: 67 - DNA, 20 bp, synthetic construct
  source 1..20: mol_type = other DNA
actgatccccataataagcg

SEQ ID NO: 68 - DNA, 20 bp, synthetic construct
  source 1..20: mol_type = other DNA
cgcttattatggggatcagt

SEQ ID NO: 69 - DNA, 20 bp, synthetic construct
  source 1..20: mol_type = other DNA
gacgagttgtgcttgtagtc

SEQ ID NO: 70 - DNA, 56 bp, synthetic construct
  source 1..56: mol_type = other DNA
cagtgccaagcttgcatgcctgcaggtcgactctagagagatcaacgaccgcccag

SEQ ID NO: 71 - DNA, 40 bp, synthetic construct
  source 1..40: mol_type = other DNA
aaaaaaacgcggagaaattcttagatcttggccggagcca

SEQ ID NO: 72 - DNA, 40 bp, synthetic construct
  source 1..40: mol_type = other DNA
tggctccggccaagatctaagaatttctccgcgttttttt

SEQ ID NO: 73 - DNA, 40 bp, synthetic construct
  source 1..40: mol_type = other DNA
taaagcagttcaatagccatttttccgaggtccttgttgc

SEQ ID NO: 74 - DNA, 40 bp, synthetic construct
  source 1..40: mol_type = other DNA
gcaacaaggacctcggaaaaatggctattgaactgcttta

SEQ ID NO: 75 - DNA, 58 bp, synthetic construct
  source 1..58: mol_type = other DNA
cagctatgaccatgattacgaattcgagctcggtaccctgaggcgcttggtgaaggtg

SEQ ID NO: 76 - DNA, 40 bp, synthetic construct
  source 1..40: mol_type = other DNA
aaaaaaacgcgaagaaattcttagatcttggccggagcca

SEQ ID NO: 77 - DNA, 40 bp, synthetic construct
  source 1..40: mol_type = other DNA
tggctccggccaagatctaagaatttcttcgcgttttttt

SEQ ID NO: 78 - DNA, 40 bp, synthetic construct
  source 1..40: mol_type = other DNA
taaagcagttcaatagccatgatttggaggtccctgcgtt

SEQ ID NO: 79 - DNA, 40 bp, synthetic construct
  source 1..40: mol_type = other DNA
aacgcagggacctccaaatcatggctattgaactgcttta

SEQ ID NO: 80 - DNA, 20 bp, synthetic construct
  source 1..20: mol_type = other DNA
cccgactttgttaccctttc

SEQ ID NO: 81 - DNA, 20 bp, synthetic construct
  source 1..20: mol_type = other DNA
actgatccccataataagcg

SEQ ID NO: 82 - DNA, 20 bp, synthetic construct
  source 1..20: mol_type = other DNA
cgcttattatggggatcagt

SEQ ID NO: 83 - DNA, 20 bp, synthetic construct
  source 1..20: mol_type = other DNA
gggtggttgttgtaggaagc